European Patent Specification EP 4 125 379 B1, published August 21, 2024. Title: Anti-Fungal Polypeptides. Applicant: Biotalys N.V. The sequence listing filed with the application follows.

SEQUENCE LISTING (161 sequences)

SEQ ID NO: 1 - protein, 119 aa, artificial sequence
  10G11Q
QVQLVESGGGLVQAGGSLRLSCAASRSIFSINAMDWYRQAPGKQREWVAGITRGGTTKYADSVKGRFTISRDNAKKKVYLQMNSLKPEDTAVYYCNVLRGEQPWTRDYWGQGTQVTVSS

SEQ ID NO: 2 - protein, 119 aa, artificial sequence
  10G11
DVQLVESGGGLVQAGGSLRLSCAASRSIFSINAMDWYRQAPGKQREWVAGITRGGTTKYADSVKGRFTISRDNAKKKVYLQMNSLKPEDTAVYYCNVLRGEQPWTRDYWGQGTQVTVSS

SEQ ID NO: 3 - protein, 117 aa, artificial sequence
  10E11Q
QVQLQESGGGLVQAGGSLRLSCAASGTIFRPTAMGWYRQAPGKERELVATITTGGSTKYADSVKGRFTISRGNAKNTVYLQMSSLKPEDTAVYYCNAQWGVRTRDYWGQGTQVTVSS

SEQ ID NO: 4 - protein, 117 aa, artificial sequence
  10E11
DVQLQESGGGLVQAGGSLRLSCAASGTIFRPTAMGWYRQAPGKERELVATITTGGSTKYADSVKGRFTISRGNAKNTVYLQMSSLKPEDTAVYYCNAQWGVRTRDYWGQGTQVTVSS

SEQ ID NO: 5 - protein, 126 aa, artificial sequence
  12C03Q
QVQLQESGGGLVQAGDSLRLSCAASISDRAFSRHVMGWFRQPPGKEREFVAAIGWTGRRTYYADSVKGRFTISRDNAMNTVYLQMNSLKPEDTAVYYCAASHFYSVSFEINDYDYWGQGTQVTVSS

SEQ ID NO: 6 - protein, 126 aa, artificial sequence
  12C03
DVQLQESGGGLVQAGDSLRLSCAASISDRAFSRHVMGWFRQPPGKEREFVAAIGWTGRRTYYADSVKGRFTISRDNAMNTVYLQMNSLKPEDTAVYYCAASHFYSVSFEINDYDYWGQGTQVTVSS

SEQ ID NO: 7 - protein, 119 aa, artificial sequence
  Mutant 1
DVQLVESGGGLVQAGGSLRLSCAASASIFSINAMDWYRQAPGKQREWVAGITRGGTTKYADSVKGRFTISRDNAKKKVYLQMNSLKPEDTAVYYCNVLRGEQPWTRDYWGQGTQVTVSS

SEQ ID NO: 8 - protein, 119 aa, artificial sequence
  Mutant 2
DVQLVESGGGLVQAGGSLRLSCAASRSIFSINAMDWYRQAPGKQREWVAGITAGGTTAYADSVKGRFTISRDNAKKKVYLQMNSLKPEDTAVYYCNVLRGEQPWTRDYWGQGTQVTVSS

SEQ ID NO: 9 - protein, 119 aa, artificial sequence
  Mutant 3
DVQLVESGGGLVQAGGSLRLSCAASRSIFSINAMDWYRQAPGKQREWVAGITRGGTTKYADSVKGRFTISRDNAKKKVYLQMNSLKPEDTAVYYCNVLAGEQPWTADYWGQGTQVTVSS

SEQ ID NO: 10 - protein, 119 aa, artificial sequence
  Mutant 4
DVQLVESGGGLVQAGGSLRLSCAASASIFSINAMDWYRQAPGKQREWVAGITAGGTTAYADSVKGRFTISRDNAKKKVYLQMNSLKPEDTAVYYCNVLAGEQPWTADYWGQGTQVTVSS

SEQ ID NO: 11 - protein, 119 aa, artificial sequence
  Mutant 5
DVQLVESGGGLVQAGGSLRLSCAASASIFSINAMDWYRQAPGKQREWVAGITAGGTTAYADSVKGRFTISRDNAKNTVYLQMNSLKPEDTAVYYCNVLAGEQPWTADYWGQGTQVTVSS

SEQ ID NO: 12 - protein, 119 aa, artificial sequence
  Mutant 6
DVQLVESGGGLVQAGGSLRLSCAASRHHFHINAMDWYRQAPGKQREWVAGITRGGTTKYADSVKGRFTISRDNAKKKVYLQMNSLKPEDTAVYYCNVLRGEQPWTRDYWGQGTQVTVSS

SEQ ID NO: 13 - protein, 119 aa, artificial sequence
  Mutant 7
DVQLVESGGGLVQAGGSLRLSCAASRSIFSINAMDWYRQAPGKQREWVAGITRGGTTKYADSVKGRFTISRDNAKKKVYLQMNSLKPEDTAVYYCNVLRGEQPHHRDYWGQGTQVTVSS

SEQ ID NO: 14 - protein, 119 aa, artificial sequence
  Mutant 8
DVQLVESGGGLVQAGGSLRLSCAASRHHFHINAMDWYRQAPGKQREWVAGITRGGTTKYADSVKGRFTISRDNAKKKVYLQMNSLKPEDTAVYYCNVLRGEQPHHRDYWGQGTQVTVSS

SEQ ID NO: 15 - protein, 119 aa, artificial sequence
  Mutant 9
DVQLVESGGGLVQAGGSLRLSCAASRKKFKINAMDWYRQAPGKQREWVAGITRGGTTKYADSVKGRFTISRDNAKKKVYLQMNSLKPEDTAVYYCNVLRGEQPWTRDYWGQGTQVTVSS

SEQ ID NO: 16 - protein, 119 aa, artificial sequence
  Mutant 10
DVQLVESGGGLVQAGGSLRLSCAASRSIFSINAMDWYRQAPGKQREWVAGITRGGTTKYADSVKGRFTISRDNAKKKVYLQMNSLKPEDTAVYYCNVLRGEQPKKRDYWGQGTQVTVSS

SEQ ID NO: 17 - protein, 119 aa, artificial sequence
  Mutant 11
DVQLVESGGGLVQAGGSLRLSCAASRKKFKINAMDWYRQAPGKQREWVAGITRGGTTKYADSVKGRFTISRDNAKKKVYLQMNSLKPEDTAVYYCNVLRGEQPKKRDYWGQGTQVTVSS

SEQ ID NO: 18 - protein, 119 aa, artificial sequence
  Single ALA mutant 1
DVQLVESGGGLVQAGGSLRLSCAASGSIFSINAMDWYRQAPGKQREWVAGITRGGTTKYADSVKGRFTISRDNAKKKVYLQMNSLKPEDTAVYYCNVLRGEQPWTRDYWGQGTQVTVSS

SEQ ID NO: 19 - protein, 119 aa, artificial sequence
  Single ALA mutant 2
DVQLVESGGGLVQAGGSLRLSCAASRAIFSINAMDWYRQAPGKQREWVAGITRGGTTKYADSVKGRFTISRDNAKKKVYLQMNSLKPEDTAVYYCNVLRGEQPWTRDYWGQGTQVTVSS

SEQ ID NO: 20 - protein, 119 aa, artificial sequence
  Single ALA mutant 3
DVQLVESGGGLVQAGGSLRLSCAASRSAFSINAMDWYRQAPGKQREWVAGITRGGTTKYADSVKGRFTISRDNAKKKVYLQMNSLKPEDTAVYYCNVLRGEQPWTRDYWGQGTQVTVSS

SEQ ID NO: 21 - protein, 119 aa, artificial sequence
  Single ALA mutant 4
DVQLVESGGGLVQAGGSLRLSCAASRSIASINAMDWYRQAPGKQREWVAGITRGGTTKYADSVKGRFTISRDNAKKKVYLQMNSLKPEDTAVYYCNVLRGEQPWTRDYWGQGTQVTVSS

SEQ ID NO: 22 - protein, 119 aa, artificial sequence
  Single ALA mutant 5
DVQLVESGGGLVQAGGSLRLSCAASRSIFAINAMDWYRQAPGKQREWVAGITRGGTTKYADSVKGRFTISRDNAKKKVYLQMNSLKPEDTAVYYCNVLRGEQPWTRDYWGQGTQVTVSS

SEQ ID NO: 23 - protein, 119 aa, artificial sequence
  Single ALA mutant 6
DVQLVESGGGLVQAGGSLRLSCAASRSIFSANAMDWYRQAPGKQREWVAGITRGGTTKYADSVKGRFTISRDNAKKKVYLQMNSLKPEDTAVYYCNVLRGEQPWTRDYWGQGTQVTVSS

SEQ ID NO: 24 - protein, 119 aa, artificial sequence
  Single ALA mutant 7
DVQLVESGGGLVQAGGSLRLSCAASRSIFSIAAMDWYRQAPGKQREWVAGITRGGTTKYADSVKGRFTISRDNAKKKVYLQMNSLKPEDTAVYYCNVLRGEQPWTRDYWGQGTQVTVSS

SEQ ID NO: 25 - protein, 119 aa, artificial sequence
  Single ALA mutant 8
DVQLVESGGGLVQAGGSLRLSCAASRSIFSINAADWYRQAPGKQREWVAGITRGGTTKYADSVKGRFTISRDNAKKKVYLQMNSLKPEDTAVYYCNVLRGEQPWTRDYWGQGTQVTVSS

SEQ ID NO: 26 - protein, 119 aa, artificial sequence
  Single ALA mutant 9
DVQLVESGGGLVQAGGSLRLSCAASRSIFSINAMAWYRQAPGKQREWVAGITRGGTTKYADSVKGRFTISRDNAKKKVYLQMNSLKPEDTAVYYCNVLRGEQPWTRDYWGQGTQVTVSS

SEQ ID NO: 27 - protein, 119 aa, artificial sequence
  Single ALA mutant 10
DVQLVESGGGLVQAGGSLRLSCAASRSIFSINAMGWYRQAPGKQREWVAGITRGGTTKYADSVKGRFTISRDNAKKKVYLQMNSLKPEDTAVYYCNVLRGEQPWTRDYWGQGTQVTVSS

SEQ ID NO: 28 - protein, 119 aa, artificial sequence
  Single ALA mutant 11
DVQLVESGGGLVQAGGSLRLSCAASRSIFSINAMDWYRQAPGKQREWVAAITRGGTTKYADSVKGRFTISRDNAKKKVYLQMNSLKPEDTAVYYCNVLRGEQPWTRDYWGQGTQVTVSS

SEQ ID NO: 29 - protein, 119 aa, artificial sequence
  Single ALA mutant 12
DVQLVESGGGLVQAGGSLRLSCAASRSIFSINAMDWYRQAPGKQREWVAGATRGGTTKYADSVKGRFTISRDNAKKKVYLQMNSLKPEDTAVYYCNVLRGEQPWTRDYWGQGTQVTVSS

SEQ ID NO: 30 - protein, 119 aa, artificial sequence
  Single ALA mutant 13
DVQLVESGGGLVQAGGSLRLSCAASRSIFSINAMDWYRQAPGKQREWVAGIARGGTTKYADSVKGRFTISRDNAKKKVYLQMNSLKPEDTAVYYCNVLRGEQPWTRDYWGQGTQVTVSS

SEQ ID NO: 31 - protein, 119 aa, artificial sequence
  Single ALA mutant 14
DVQLVESGGGLVQAGGSLRLSCAASRSIFSINAMDWYRQAPGKQREWVAGITAGGTTKYADSVKGRFTISRDNAKKKVYLQMNSLKPEDTAVYYCNVLRGEQPWTRDYWGQGTQVTVSS

SEQ ID NO: 32 - protein, 119 aa, artificial sequence
  Single ALA mutant 15
DVQLVESGGGLVQAGGSLRLSCAASRSIFSINAMDWYRQAPGKQREWVAGITSGGTTKYADSVKGRFTISRDNAKKKVYLQMNSLKPEDTAVYYCNVLRGEQPWTRDYWGQGTQVTVSS

SEQ ID NO: 33 - protein, 119 aa, artificial sequence
  Single ALA mutant 16
DVQLVESGGGLVQAGGSLRLSCAASRSIFSINAMDWYRQAPGKQREWVAGITRAGTTKYADSVKGRFTISRDNAKKKVYLQMNSLKPEDTAVYYCNVLRGEQPWTRDYWGQGTQVTVSS

SEQ ID NO: 34 - protein, 119 aa, artificial sequence
  Single ALA mutant 17
DVQLVESGGGLVQAGGSLRLSCAASRSIFSINAMDWYRQAPGKQREWVAGITRGATTKYADSVKGRFTISRDNAKKKVYLQMNSLKPEDTAVYYCNVLRGEQPWTRDYWGQGTQVTVSS

SEQ ID NO: 35 - protein, 119 aa, artificial sequence
  Single ALA mutant 18
DVQLVESGGGLVQAGGSLRLSCAASRSIFSINAMDWYRQAPGKQREWVAGITRGGATKYADSVKGRFTISRDNAKKKVYLQMNSLKPEDTAVYYCNVLRGEQPWTRDYWGQGTQVTVSS

SEQ ID NO: 36 - protein, 119 aa, artificial sequence
  Single ALA mutant 19
DVQLVESGGGLVQAGGSLRLSCAASRSIFSINAMDWYRQAPGKQREWVAGITRGGSTKYADSVKGRFTISRDNAKKKVYLQMNSLKPEDTAVYYCNVLRGEQPWTRDYWGQGTQVTVSS

SEQ ID NO: 37 - protein, 119 aa, artificial sequence
  Single ALA mutant 20
DVQLVESGGGLVQAGGSLRLSCAASRSIFSINAMDWYRQAPGKQREWVAGITRGGTAKYADSVKGRFTISRDNAKKKVYLQMNSLKPEDTAVYYCNVLRGEQPWTRDYWGQGTQVTVSS

SEQ ID NO: 38 - protein, 119 aa, artificial sequence
  Single ALA mutant 21
DVQLVESGGGLVQAGGSLRLSCAASRSIFSINAMDWYRQAPGKQREWVAGITRGGTTAYADSVKGRFTISRDNAKKKVYLQMNSLKPEDTAVYYCNVLRGEQPWTRDYWGQGTQVTVSS

SEQ ID NO: 39 - protein, 119 aa, artificial sequence
  Single ALA mutant 22
DVQLVESGGGLVQAGGSLRLSCAASRSIFSINAMDWYRQAPGKQREWVAGITRGGTTNYADSVKGRFTISRDNAKKKVYLQMNSLKPEDTAVYYCNVLRGEQPWTRDYWGQGTQVTVSS

SEQ ID NO: 40 - protein, 119 aa, artificial sequence
  Single ALA mutant 23
DVQLVESGGGLVQAGGSLRLSCAASRSIFSINAMDWYRQAPGKQREWVAGITRGGTTKYADSVKGRFTISRDNAKKKVYLQMNSLKPEDTAVYYCNALRGEQPWTRDYWGQGTQVTVSS

SEQ ID NO: 41 - protein, 119 aa, artificial sequence
  Single ALA mutant 24
DVQLVESGGGLVQAGGSLRLSCAASRSIFSINAMDWYRQAPGKQREWVAGITRGGTTKYADSVKGRFTISRDNAKKKVYLQMNSLKPEDTAVYYCNVARGEQPWTRDYWGQGTQVTVSS

SEQ ID NO: 42 - protein, 119 aa, artificial sequence
  Single ALA mutant 25
DVQLVESGGGLVQAGGSLRLSCAASRSIFSINAMDWYRQAPGKQREWVAGITRGGTTKYADSVKGRFTISRDNAKKKVYLQMNSLKPEDTAVYYCNVLAGEQPWTRDYWGQGTQVTVSS

SEQ ID NO: 43 - protein, 119 aa, artificial sequence
  Single ALA mutant 26
DVQLVESGGGLVQAGGSLRLSCAASRSIFSINAMDWYRQAPGKQREWVAGITRGGTTKYADSVKGRFTISRDNAKKKVYLQMNSLKPEDTAVYYCNVLRAEQPWTRDYWGQGTQVTVSS

SEQ ID NO: 44 - protein, 119 aa, artificial sequence
  Single ALA mutant 27
DVQLVESGGGLVQAGGSLRLSCAASRSIFSINAMDWYRQAPGKQREWVAGITRGGTTKYADSVKGRFTISRDNAKKKVYLQMNSLKPEDTAVYYCNVLRGAQPWTRDYWGQGTQVTVSS

SEQ ID NO: 45 - protein, 119 aa, artificial sequence
  Single ALA mutant 28
DVQLVESGGGLVQAGGSLRLSCAASRSIFSINAMDWYRQAPGKQREWVAGITRGGTTKYADSVKGRFTISRDNAKKKVYLQMNSLKPEDTAVYYCNVLRGEAPWTRDYWGQGTQVTVSS

SEQ ID NO: 46 - protein, 119 aa, artificial sequence
  Single ALA mutant 29
DVQLVESGGGLVQAGGSLRLSCAASRSIFSINAMDWYRQAPGKQREWVAGITRGGTTKYADSVKGRFTISRDNAKKKVYLQMNSLKPEDTAVYYCNVLRGEQAWTRDYWGQGTQVTVSS

SEQ ID NO: 47 - protein, 119 aa, artificial sequence
  Single ALA mutant 30
DVQLVESGGGLVQAGGSLRLSCAASRSIFSINAMDWYRQAPGKQREWVAGITRGGTTKYADSVKGRFTISRDNAKKKVYLQMNSLKPEDTAVYYCNVLRGEQPATRDYWGQGTQVTVSS

SEQ ID NO: 48 - protein, 119 aa, artificial sequence
  Single ALA mutant 31
DVQLVESGGGLVQAGGSLRLSCAASRSIFSINAMDWYRQAPGKQREWVAGITRGGTTKYADSVKGRFTISRDNAKKKVYLQMNSLKPEDTAVYYCNVLRGEQPWARDYWGQGTQVTVSS

SEQ ID NO: 49 - protein, 119 aa, artificial sequence
  Single ALA mutant 32
DVQLVESGGGLVQAGGSLRLSCAASRSIFSINAMDWYRQAPGKQREWVAGITRGGTTKYADSVKGRFTISRDNAKKKVYLQMNSLKPEDTAVYYCNVLRGEQPWTADYWGQGTQVTVSS

SEQ ID NO: 50 - protein, 119 aa, artificial sequence
  Single ALA mutant 33
DVQLVESGGGLVQAGGSLRLSCAASRSIFSINAMDWYRQAPGKQREWVAGITRGGTTKYADSVKGRFTISRDNAKKKVYLQMNSLKPEDTAVYYCNVLRGEQPWTRAYWGQGTQVTVSS

SEQ ID NO: 51 - protein, 119 aa, artificial sequence
  Single ALA mutant 34
DVQLVESGGGLVQAGGSLRLSCAASRSIFSINAMDWYRQAPGKQREWVAGITRGGTTKYADSVKGRFTISRDNAKKKVYLQMNSLKPEDTAVYYCNVLRGEQPWTRDAWGQGTQVTVSS

SEQ ID NO: 52 - protein, 10 aa, artificial sequence
  CDR1-10G11 (and CDR1-10G11Q)
RSIFSINAMD

SEQ ID NO: 53 - protein, 10 aa, artificial sequence
  CDR1-10E11 (and CDR1-10E11Q)
GTIFRPTAMG

SEQ ID NO: 54 - protein, 10 aa, artificial sequence
  CDR1-12C03 (and CDR1-12C03Q)
ISDRAFSRHV

SEQ ID NO: 55 - protein, 10 aa, artificial sequence
  CDR1-Mutant 1
ASIFSINAMD

SEQ ID NO: 56 - protein, 10 aa, artificial sequence
  CDR1-Mutant 6 and 8
RHHFHINAMD

SEQ ID NO: 57 - protein, 10 aa, artificial sequence
  CDR1-Mutant 9 and 11
RKKFKINAMD

SEQ ID NO: 58 - protein, 10 aa, artificial sequence
  CDR1-Single ALA mutant 1
GSIFSINAMD

SEQ ID NO: 59 - protein, 10 aa, artificial sequence
  CDR1-Single ALA mutant 2
RAIFSINAMD

SEQ ID NO: 60 - protein, 10 aa, artificial sequence
  CDR1-Single ALA mutant 3
RSAFSINAMD

SEQ ID NO: 61 - protein, 10 aa, artificial sequence
  CDR1-Single ALA mutant 4
RSIASINAMD

SEQ ID NO: 62 - protein, 10 aa, artificial sequence
  CDR1-Single ALA mutant 5
RSIFAINAMD

SEQ ID NO: 63 - protein, 10 aa, artificial sequence
  CDR1-Single ALA mutant 6
RSIFSANAMD

SEQ ID NO: 64 - protein, 10 aa, artificial sequence
  CDR1-Single ALA mutant 7
RSIFSIAAMD

SEQ ID NO: 65 - protein, 10 aa, artificial sequence
  CDR1-Single ALA mutant 8
RSIFSINAAD

SEQ ID NO: 66 - protein, 10 aa, artificial sequence
  CDR1-Single ALA mutant 9
RSIFSINAMA

SEQ ID NO: 67 - protein, 10 aa, artificial sequence
  CDR1-Single ALA mutant 10
RSIFSINAMG

SEQ ID NO: 68 - protein, 9 aa, artificial sequence
  CDR2-10G11 (and CDR2-10G11Q)
GITRGGTTK

SEQ ID NO: 69 - protein, 9 aa, artificial sequence
  CDR2-10E11 (and CDR2-10E11Q)
TITTGGSTK

SEQ ID NO: 70 - protein, 10 aa, artificial sequence
  CDR2-12C03 (and CDR2-12C03Q)
AIGWTGRRTY

SEQ ID NO: 71 - protein, 9 aa, artificial sequence
  CDR2-Mutant 2
GITAGGTTA

SEQ ID NO: 72 - protein, 9 aa, artificial sequence
  CDR2-Single ALA mutant 11
AITRGGTTK

SEQ ID NO: 73 - protein, 9 aa, artificial sequence
  CDR2-Single ALA mutant 12
GATRGGTTK

SEQ ID NO: 74 - protein, 9 aa, artificial sequence
  CDR2-Single ALA mutant 13
GIARGGTTK

SEQ ID NO: 75 - protein, 9 aa, artificial sequence
  CDR2-Single ALA mutant 14
GITAGGTTK

SEQ ID NO: 76 - protein, 9 aa, artificial sequence
  CDR2-Single ALA mutant 15
GITSGGTTK

SEQ ID NO: 77 - protein, 9 aa, artificial sequence
  CDR2-Single ALA mutant 16
GITRAGTTK

SEQ ID NO: 78 - protein, 9 aa, artificial sequence
  CDR2-Single ALA mutant 17
GITRGATTK

SEQ ID NO: 79 - protein, 9 aa, artificial sequence
  CDR2-Single ALA mutant 18
GITRGGATK

SEQ ID NO: 80 - protein, 9 aa, artificial sequence
  CDR2-Single ALA mutant 19
GITRGGSTK

SEQ ID NO: 81 - protein, 9 aa, artificial sequence
  CDR2-Single ALA mutant 20
GITRGGTAK

SEQ ID NO: 82 - protein, 9 aa, artificial sequence
  CDR2-Single ALA mutant 21
GITRGGTTA

SEQ ID NO: 83 - protein, 9 aa, artificial sequence
  CDR2-Single ALA mutant 22
GITRGGTTN

SEQ ID NO: 84 - protein, 11 aa, artificial sequence
  CDR3-10G11 (and CDR3-10G11Q)
LRGEQPWTRDY

SEQ ID NO: 85 - protein, 9 aa, artificial sequence
  CDR3-10E11 (and CDR3-10E11Q)
QWGVRTRDY

SEQ ID NO: 86 - protein, 15 aa, artificial sequence
  CDR3-12C03 (and CDR3-12C03Q)
SHFYSVSFEINDYDY

SEQ ID NO: 87 - protein, 11 aa, artificial sequence
  CDR3-Mutant 3
LAGEQPWTADY

SEQ ID NO: 88 - protein, 11 aa, artificial sequence
  CDR3-Mutant 7
LRGEQPHHRDY

SEQ ID NO: 89 - protein, 11 aa, artificial sequence
  CDR3-Mutant 10
LRGEQPKKRDY

SEQ ID NO: 90 - protein, 11 aa, artificial sequence
  CDR3-Single ALA mutant 24
ARGEQPWTRDY

SEQ ID NO: 91 - protein, 11 aa, artificial sequence
  CDR3-Single ALA mutant 25
LAGEQPWTRDY

SEQ ID NO: 92 - protein, 11 aa, artificial sequence
  CDR3-Single ALA mutant 26
LRAEQPWTRDY

SEQ ID NO: 93 - protein, 11 aa, artificial sequence
  CDR3-Single ALA mutant 27
LRGAQPWTRDY

SEQ ID NO: 94 - protein, 11 aa, artificial sequence
  CDR3-Single ALA mutant 28
LRGEAPWTRDY

SEQ ID NO: 95 - protein, 11 aa, artificial sequence
  CDR3-Single ALA mutant 29
LRGEQAWTRDY

SEQ ID NO: 96 - protein, 11 aa, artificial sequence
  CDR3-Single ALA mutant 30
LRGEQPATRDY

SEQ ID NO: 97 - protein, 11 aa, artificial sequence
  CDR3-Single ALA mutant 31
LRGEQPWARDY

SEQ ID NO: 98 - protein, 11 aa, artificial sequence
  CDR3-Single ALA mutant 32
LRGEQPWTADY

SEQ ID NO: 99 - protein, 11 aa, artificial sequence
  CDR3-Single ALA mutant 33
LRGEQPWTRAY

SEQ ID NO: 100 - protein, 11 aa, artificial sequence
  CDR3-Single ALA mutant 34
LRGEQPWTRDA

SEQ ID NO: 101 - protein, 119 aa, artificial sequence
  10G11 General Formula A
  misc_feature (1)..(1): X is D or Q
  misc_feature (26)..(28): X is G, A, V, L, I, M, P, F, W, S, T, N, Q, Y, C, K, R, H, D or E
  misc_feature (30)..(30): X is G, A, V, L, I, M, P, F, W, S, T, N, Q, Y, C, K, R, H, D or E
  misc_feature (53)..(53): X is G, A, V, L, I, M, P, F, W, S, T, N, Q, Y, C, K, R, H, D or E
  misc_feature (58)..(58): X is G, A, V, L, I, M, P, F, W, S, T, N, Q, Y, C, K, R, H, D or E
  misc_feature (99)..(99): X is G, A, V, L, I, M, P, F, W, S, T, N, Q, Y, C, K, R, H, D or E
  misc_feature (104)..(106): X is G, A, V, L, I, M, P, F, W, S, T, N, Q, Y, C, K, R, H, D or E
XVQLVESGGGLVQAGGSLRLSCAASXXXFXINAMDWYRQAPGKQREWVAGITXGGTTXYADSVKGRFTISRDNAKKKVYLQMNSLKPEDTAVYYCNVLXGEQPXXXDYWGQGTQVTVSS

SEQ ID NO: 102 - protein, 119 aa, artificial sequence; identical to SEQ ID NO: 101
  10G11 General Formula B
  misc_feature (1)..(1): X is D or Q
  misc_feature (26)..(28): X is G, A, V, L, I, M, P, F, W, S, T, N, Q, Y, C, K, R or H
  misc_feature (30)..(30): X is G, A, V, L, I, M, P, F, W, S, T, N, Q, Y, C, K, R or H
  misc_feature (53)..(53): X is G, A, V, L, I, M, P, F, W, S, T, N, Q, Y, C, K, R or H
  misc_feature (58)..(58): X is G, A, V, L, I, M, P, F, W, S, T, N, Q, Y, C, K, R or H
  misc_feature (99)..(99): X is G, A, V, L, I, M, P, F, W, S, T, N, Q, Y, C, K, R or H
  misc_feature (104)..(106): X is G, A, V, L, I, M, P, F, W, S, T, N, Q, Y, C, K, R or H

SEQ ID NO: 103 - protein, 119 aa, artificial sequence; identical to SEQ ID NO: 101
  10G11 General Formula  C
  misc_feature (1)..(1): X is D or Q
  misc_feature (26)..(26): X is G, A, V, M, L, I, K, R or H
  misc_feature (27)..(28): X is G, A, V, L, I, M, P, F, W, S, T, N, Q, Y, C, K, R or H
  misc_feature (27)..(28): X is G, A, V, L, I, M, P, F, W, S, T, N, Q, Y, C, K, R or H
  misc_feature (30)..(30): X is G, A, V, L, I, M, P, F, W, S, T, N, Q, Y, C, K, R or H
  misc_feature (53)..(53): X is G, A, V, M, L, I, K, R, H
  misc_feature (58)..(58): X is G, A, V, M, L, I, K, R, H
  misc_feature (99)..(99): X is G, A, V, M, L, I, K, R, or H
  misc_feature (104)..(105): X is G, A, V, L, I, M, P, F, W, S, T, N, Q, Y, C, K, R or H
  misc_feature (106)..(106): X is G, A, V, M, L, I, K, R, or H

SEQ ID NO: 104 - protein, 119 aa, artificial sequence; identical to SEQ ID NO: 101
  10G11 General Formula D
  misc_feature (1)..(1): X is D or Q
  misc_feature (26)..(26): X is A, K, R or H
  misc_feature (27)..(28): Xaa can be any naturally occurring amino acid
  misc_feature (30)..(30): X is G, A, V, L, I, M, P, F, W, S, T, N, Q, Y, C, K, R or H
  misc_feature (53)..(53): X is A, R, K or H
  misc_feature (53)..(53): X is A, R, K or H
  misc_feature (58)..(58): X is A, R, K or H
  misc_feature (99)..(99): X is A, R, K or H
  misc_feature (104)..(105): X is G, A, V, L, I, M, P, F, W, S, T, N, Q, Y, C, K, R or H
  misc_feature (106)..(106): X is A, R, K or H

SEQ ID NO: 105 - protein, 119 aa, artificial sequence; identical to SEQ ID NO: 101
  10G11 General Formula E
  misc_feature (1)..(1): X is D or Q
  misc_feature (26)..(26): X is A, R, K, H
  misc_feature (27)..(27): X is S, T, C, P, N, Q, R or H
  misc_feature (28)..(28): X is I, G, A, V, M, L, K, R,  or H
  misc_feature (30)..(30): Xaa can be any naturally occurring amino acid
  misc_feature (53)..(53): X is S, T, C, P, N, Q, K, R or H
  misc_feature (58)..(58): X is A, K, R or H
  misc_feature (58)..(58): X is A, K, R or H
  misc_feature (99)..(99): X is A, K, R or H
  misc_feature (104)..(99): X is W, F, Y, K, R or H
  misc_feature (104)..(104): Xaa can be any naturally occurring amino acid
  misc_feature (105)..(105): X is S, T, C, P, N, Q, K, R or H
  misc_feature (106)..(106): X is A, K, R or H

SEQ ID NO: 106 - protein, 119 aa, artificial sequence; identical to SEQ ID NO: 101
  10G11 General Formula F
  misc_feature (1)..(1): X is D or Q
  misc_feature (26)..(26): X is A, K, R, H
  misc_feature (27)..(27): X is S, K, R, H
  misc_feature (28)..(28): X is I, K, R, H
  misc_feature (30)..(30): X is S, K, R, H
  misc_feature (53)..(53): X is A, K, R, H
  misc_feature (58)..(58): X is A, K, R, H
  misc_feature (99)..(99): X is A, K, R, H
  misc_feature (104)..(104): X is W, K, R, H
  misc_feature (105)..(105): X is T, K, R, H
  misc_feature (106)..(106): X is A, K, R, H

SEQ ID NO: 107 - protein, 119 aa, artificial sequence; identical to SEQ ID NO: 101
  10G11 General Formula G
  misc_feature (1)..(1): X is D or Q
  misc_feature (26)..(26): X is K, R, H
  misc_feature (27)..(7): X is S, K, R, H
  misc_feature (27)..(27): Xaa can be any naturally occurring amino acid
  misc_feature (28)..(28): X is I, K, R, H
  misc_feature (30)..(30): X is S, K, R, H
  misc_feature (53)..(53): X is K, R, H
  misc_feature (58)..(58): X is K, R, H
  misc_feature (99)..(99): X is K, R, H
  misc_feature (104)..(104): X is W, K, R, H
  misc_feature (105)..(105): X is T, K, R, H
  misc_feature (106)..(106): X is A, K, R, H

SEQ ID NO: 108 - protein, 119 aa, artificial sequence; identical to SEQ ID NO: 101
  10G11 General Formula H
  misc_feature (1)..(1): X is D or Q
  misc_feature (26)..(26): X is R
  misc_feature (27)..(28): X is R
  misc_feature (30)..(30): X is G, A, V, L, I, M, P, F, W, S, T, N, Q, Y, C, K, R, H, D, E
  misc_feature (53)..(53): X is R
  misc_feature (58)..(58): X is K
  misc_feature (99)..(99): X is R
  misc_feature (104)..(105): X is G, A, V, L, I, M, P, F, W, S, T, N, Q, Y, C, K, R, H, D, E
  misc_feature (106)..(106): X is R

SEQ ID NO: 109 - protein, 119 aa, artificial sequence; identical to SEQ ID NO: 101
  10G11 General Formula I
  misc_feature (1)..(1): X is D or Q
  misc_feature (26)..(26): X is R
  misc_feature (27)..(28): X is G, A, V, L, I, M, P, F, W, S, T, N, Q, Y, C, K, R or H
  misc_feature (30)..(30): X is G, A, V, L, I, M, P, F, W, S, T, N, Q, Y, C, K, R or H
  misc_feature (53)..(53): X is R
  misc_feature (58)..(58): X is K
  misc_feature (99)..(99): X is R
  misc_feature (104)..(105): X is G, A, V, L, I, M, P, F, W, S, T, N, Q, Y, C, K, R or H
  misc_feature (106)..(106): X is R

SEQ ID NO: 110 - protein, 119 aa, artificial sequence; identical to SEQ ID NO: 101
  10G11 General Formula J
  misc_feature (1)..(1): X is D or Q
  misc_feature (26)..(26): X is R
  misc_feature (27)..(27): X is S, T, C, P, N, Q, K, R, H
  misc_feature (28)..(28): X is I, G, A, V, M, L, K, R, H
  misc_feature (28)..(28): X is I, G, A, V, M, L, K, R, H
  misc_feature (30)..(30): X is S, T, C, P, N, Q, K, R, H
  misc_feature (53)..(53): X is R
  misc_feature (58)..(58): X is K
  misc_feature (99)..(99): X is R
  misc_feature (104)..(99): X is W, F, Y, K, R, H
  misc_feature (104)..(104): Xaa can be any naturally occurring amino acid
  misc_feature (105)..(105): X is S, T, C, P, N, Q, K, R, H
  misc_feature (106)..(106): X is R

SEQ ID NO: 111 - protein, 119 aa, artificial sequence; identical to SEQ ID NO: 101
  10G11 General Formula K
  misc_feature (1)..(1): X is D or Q
  misc_feature (10)..(106): X is R
  misc_feature (26)..(26): X is R
  misc_feature (27)..(27): X is S, K, R, H
  misc_feature (28)..(28): X is I, K, R, H
  misc_feature (30)..(30): X is S, K, R, H
  misc_feature (53)..(53): X is R
  misc_feature (58)..(58): X is K
  misc_feature (99)..(99): X is R
  misc_feature (104)..(104): X is W, K, R, H
  misc_feature (105)..(105): X is T, K, R, H

SEQ ID NO: 112 - protein, 10 aa, artificial sequence
  10G11 General Formula CDR1 A
  misc_feature (1)..(3): X is G, A, V, L, I, M, P, F, W, S, T, N, Q, Y, C, K, R, H. D, E
  misc_feature (5)..(5): X is G, A, V, L, I, M, P, F, W, S, T, N, Q, Y, C, K, R, H. D, E
XXXFXINAMD

SEQ ID NO: 113 - protein, 10 aa, artificial sequence
  10G11 General Formula CDR1 B
  misc_feature (1)..(3): X is G, A, V, L, I, M, P, F, W, S, T, N, Q, Y, C, K, R, H
  misc_feature (5)..(5): X is G, A, V, L, I, M, P, F, W, S, T, N, Q, Y, C, K, R, H
XXXFXINAMD

SEQ ID NO: 114 - protein, 10 aa, artificial sequence
  10G11 General Formula CDR1 C
  misc_feature (1)..(1): X is G, A, V, M, L, I, K, R, H
  misc_feature (2)..(3): X is G, A, V, L, I, M, P, F, W, S, T, N, Q, Y, C, K, R or H
  misc_feature (5)..(5): X is G, A, V, L, I, M, P, F, W, S, T, N, Q, Y, C, K, R or H
XXXFXINAMD

SEQ ID NO: 115 - protein, 10 aa, artificial sequence
  10G11 General Formula CDR1 D
  misc_feature (1)..(1): X is A, K, R, H
  misc_feature (2)..(3): X is G, A, V, L, I, M, P, F, W, S, T, N, Q, Y, C, K, R, H
  misc_feature (5)..(5): X is G, A, V, L, I, M, P, F, W, S, T, N, Q, Y, C, K, R, H
XXXFXINAMD

SEQ ID NO: 116 - protein, 10 aa, artificial sequence
  10G11 General Formula CDR1 E
  misc_feature (1)..(1): X is A, K, R, H
  misc_feature (2)..(2): X is S, T, C, P, N, Q, K, R, H
  misc_feature (3)..(3): X is I, G, A, V, M, L, K, R, H
  misc_feature (5)..(5): X is S, T, C, P, N, Q, K, R, H
XXXFXINAMD

SEQ ID NO: 117 - protein, 10 aa, artificial sequence
  10G11 General Formula CDR1 F
  misc_feature (1)..(1): X is A, K, R, H
  misc_feature (2)..(2): X is S, K, R, H
  misc_feature (3)..(3): X is I, K, R, H
  misc_feature (5)..(5): X is S, K, R, H
XXXFXINAMD

SEQ ID NO: 118 - protein, 10 aa, artificial sequence
  10G11 General Formula CDR1 G
  misc_feature (1)..(1): X is K, R, H
  misc_feature (2)..(2): X is S, K, R, H
  misc_feature (3)..(3): X is I, K, R, H
  misc_feature (5)..(5): X is S, K, R, H
XXXFXINAMD

SEQ ID NO: 119 - protein, 10 aa, artificial sequence
  10G11 General Formula CDR1 H
  misc_feature (1)..(1): X is R
  misc_feature (2)..(3): X is G, A, V, L, I, M, P, F, W, S, T, N, Q, Y, C, K, R, H, D, E
  misc_feature (5)..(5): X is G, A, V, L, I, M, P, F, W, S, T, N, Q, Y, C, K, R, H, D, E
XXXFXINAMD

SEQ ID NO: 120 - protein, 10 aa, artificial sequence
  10G11 General Formula CDR1 I
  misc_feature (1)..(1): X is R
  misc_feature (2)..(3): X is G, A, V, L, I, M, P, F, W, S, T, N, Q, Y, C, K, R, H
  misc_feature (5)..(5): X is G, A, V, L, I, M, P, F, W, S, T, N, Q, Y, C, K, R, H
XXXFXINAMD

SEQ ID NO: 121 - protein, 10 aa, artificial sequence
  10G11 General Formula CDR1 J
  misc_feature (1)..(1): X is R
  misc_feature (2)..(2): X is S, T, C, P, N, Q, K, R, H
  misc_feature (3)..(3): X is I, G, A, V, M, L, K, R, H
  misc_feature (5)..(5): X is S, T, C, P, N, Q, K, R, H
XXXFXINAMD

SEQ ID NO: 122 - protein, 10 aa, artificial sequence
  10G11 General Formula CDR1 K
  misc_feature (1)..(1): X is R
  misc_feature (2)..(2): X is S, K, R, H
  misc_feature (3)..(3): X is I, K, R, H
  misc_feature (5)..(5): X is S, K, R, H
XXXFXINAMD

SEQ ID NO: 123 - protein, 9 aa, artificial sequence
  10G11 General Formula CDR2 A
  misc_feature (4)..(4): X is G, A, V, L, I, M, P, F, W, S, T, N, Q, Y, C, K, R, H, D, E
  misc_feature (9)..(9): X is G, A, V, L, I, M, P, F, W, S, T, N, Q, Y, C, K, R, H, D, E
GITXGGTTX

SEQ ID NO: 124 - protein, 9 aa, artificial sequence
  10G11 General Formula CDR2 B
  misc_feature (4)..(4): Xaa can be any naturally occurring amino acid
  misc_feature (9)..(9): X is G, A, V, L, I, M, P, F, W, S, T, N, Q, Y, C, K, R, H
GITXGGTTX

SEQ ID NO: 125 - protein, 9 aa, artificial sequence
  10G11 General Formula CDR2 C
  misc_feature (4)..(4): X is G, A, V, M, L, I, K, R, H
  misc_feature (9)..(9): X is G, A, V, M, L, I, K, R, H
GITXGGTTX

SEQ ID NO: 126 - protein, 9 aa, artificial sequence
  10G11 General Formula CDR2 D
  misc_feature (4)..(4): X is A, K, R, H
  misc_feature (9)..(9): X is A, K, R, H
GITXGGTTX

SEQ ID NO: 127 - protein, 9 aa, artificial sequence
  10G11 General Formula CDR2 E
  misc_feature (4)..(4): X is A, K, R, H
  misc_feature (9)..(9): X is A, K, R, H
GITXGGTTX

SEQ ID NO: 128 - protein, 9 aa, artificial sequence
  10G11 General Formula CDR2 F
  misc_feature (4)..(4): X is A, K, R, H
  misc_feature (9)..(9): X is A, K, R, H
GITXGGTTX

SEQ ID NO: 129 - protein, 9 aa, artificial sequence
  10G11 General Formula CDR2 G
  misc_feature (4)..(4): X is K, R, H
  misc_feature (9)..(9): X is K, R, H
GITXGGTTX

SEQ ID NO: 130 - protein, 9 aa, artificial sequence
  10G11 General Formula CDR2 H
  misc_feature (4)..(4): X is R
  misc_feature (9)..(9): X is K
GITXGGTTX

SEQ ID NO: 131 - protein, 9 aa, artificial sequence
  10G11 General Formula CDR2 I
  misc_feature (4)..(4): X is R
  misc_feature (9)..(9): X is K
GITXGGTTX

SEQ ID NO: 132 - protein, 9 aa, artificial sequence
  10G11 General Formula CDR2 J
  misc_feature (4)..(4): X is R
  misc_feature (9)..(9): X is K
GITXGGTTX

SEQ ID NO: 133 - protein, 9 aa, artificial sequence
  10G11 General Formula CDR2 K
  misc_feature (4)..(4): X is R
  misc_feature (9)..(9): X is K
GITXGGTTX

SEQ ID NO: 134 - protein, 11 aa, artificial sequence
  10G11 General Formula CDR3 A
  misc_feature (2)..(2): X is G, A, V, L, I, M, P, F, W, S, T, N, Q, Y, C, K, R, H, D, E
  misc_feature (7)..(9): X is G, A, V, L, I, M, P, F, W, S, T, N, Q, Y, C, K, R, H, D, E
LXGEQPXXXDY

SEQ ID NO: 135 - protein, 11 aa, artificial sequence
  10G11 General Formula CDR3 B
  misc_feature (2)..(2): X is X is G, A, V, L, I, M, P, F, W, S, T, N, Q, Y, C, K, R, H
  misc_feature (7)..(9): X is X is G, A, V, L, I, M, P, F, W, S, T, N, Q, Y, C, K, R, H
LXGEQPXXXDY

SEQ ID NO: 136 - protein, 11 aa, artificial sequence
  10G11 General Formula CDR3 C
  misc_feature (2)..(2): X is G, A, V, M, L, I, K, R, H
  misc_feature (7)..(8): X is G, A, V, L, I, M, P, F, W, S, T, N, Q, Y, C, K, R, H
  misc_feature (9)..(9): X is G, A, V, M, L, I, K, R, H
LXGEQPXXXDY

SEQ ID NO: 137 - protein, 11 aa, artificial sequence
  10G11 General Formula CDR3 D
  misc_feature (2)..(2): X is A, K, R, H
  misc_feature (7)..(8): X is G, A, V, L, I, M, P, F, W, S, T, N, Q, Y, C, K, R, H
  misc_feature (9)..(9): X is A, K, R, H
LXGEQPXXXDY

SEQ ID NO: 138 - protein, 11 aa, artificial sequence
  10G11 General Formula CDR3 E
  misc_feature (2)..(2): X is A, K, R, H
  misc_feature (7)..(7): X is W, F, Y, K, R, H
  misc_feature (8)..(8): X is S, T, C, P, N, Q, K, R, H
  misc_feature (9)..(9): X is A, K, R, H
LXGEQPXXXDY

SEQ ID NO: 139 - protein, 11 aa, artificial sequence
  10G11 General Formula CDR3 F
  misc_feature (2)..(2): X is A, K, R, H
  misc_feature (7)..(7): X is W, K, R, H
  misc_feature (8)..(8): X is T, K, R, H
  misc_feature (9)..(9): X is A, K, R, H
LXGEQPXXXDY

SEQ ID NO: 140 - protein, 11 aa, artificial sequence
  10G11 General Formula CDR3 G
  misc_feature (2)..(2): X is K, R, H
  misc_feature (7)..(7): X is W, K, R, H
  misc_feature (8)..(8): X is T, K, R, H
  misc_feature (9)..(9): X is K, R, H
LXGEQPXXXDY

SEQ ID NO: 141 - protein, 11 aa, artificial sequence
  10G11 General Formula CDR3 H
  misc_feature (2)..(2): X is R
  misc_feature (7)..(8): X is G, A, V, L, I, M, P, F, W, S, T, N, Q, Y, C, K, R, H, D, E
  misc_feature (9)..(9): X is R
LXGEQPXXXDY

SEQ ID NO: 142 - protein, 11 aa, artificial sequence
  10G11 General Formula CDR3 I
  misc_feature (2)..(2): X is R
  misc_feature (7)..(8): X is G, A, V, L, I, M, P, F, W, S, T, N, Q, Y, C, K, R, H
  misc_feature (9)..(9): X is R
LXGEQPXXXDY

SEQ ID NO: 143 - protein, 11 aa, artificial sequence
  10G11 General Formula CDR3 J
  misc_feature (2)..(2): X is R
  misc_feature (7)..(7): X is W, F, Y, K, R, H
  misc_feature (8)..(8): X is S, T, C, P, N, Q, K, R, H
  misc_feature (9)..(9): X is R
LXGEQPXXXDY

SEQ ID NO: 144 - protein, 11 aa, artificial sequence
  10G11 General Formula CDR3 K
  misc_feature (2)..(2): X is R
  misc_feature (7)..(7): X is W, K, R, H
  misc_feature (8)..(8): X is T, K, R, H
  misc_feature (9)..(9): X is R
LXGEQPXXXDY

SEQ ID NO: 145 - protein, 119 aa, artificial sequence
  Germline
  misc_feature (98)..(108): X is unknown
QVQLVESGGGLVQAGGSLRLSCAASGSIFSINAMGWYRQAPGKQRELVAAITSGGSTNYADSVKGRFTISRDNAKNTVYLQMNSLKPEDTAVYYCNAXXXXXXXXXXXWGQGTQVTVSS

SEQ ID NO: 146 - protein, 126 aa, artificial sequence
  10E11Q-His
QVQLQESGGGLVQAGGSLRLSCAASGTIFRPTAMGWYRQAPGKERELVATITTGGSTKYADSVKGRFTISRGNAKNTVYLQMSSLKPEDTAVYYCNAQWGVRTRDYWGQGTQVTVSSAAAHHHHHH

SEQ ID NO: 147 - protein, 135 aa, artificial sequence
  12C03Q-His
QVQLQESGGGLVQAGDSLRLSCAASISDRAFSRHVMGWFRQPPGKEREFVAAIGWTGRRTYYADSVKGRFTISRDNAMNTVYLQMNSLKPEDTAVYYCAASHFYSVSFEINDYDYWGQGTQVTVSSAAAHHHHHH

SEQ ID NO: 148 - protein, 128 aa, artificial sequence
  10G11Q-His
QVQLQESGGGLVQAGGSLRLSCAASRSIFSINAMDWYRQAPGKQREWVAGITRGGTTKYADSVKGRFTISRDNAKKKVYLQMNSLKPEDTAVYYCNVLRGEQPWTRDYWGQGTQVTVSSAAAHHHHHH

SEQ ID NO: 149 - protein, 25 aa, artificial sequence
  10G11 Framework region 1 (Q)
QVQLVESGGGLVQAGGSLRLSCAAS

SEQ ID NO: 150 - protein, 25 aa, artificial sequence
  10G11 Framework region 1 (D)
DVQLVESGGGLVQAGGSLRLSCAAS

SEQ ID NO: 151 - protein, 14 aa, artificial sequence
  10G11 Framework region 2
WYRQAPGKQREWVA

SEQ ID NO: 152 - protein, 39 aa, artificial sequence
  10G11 Framework region 3
YADSVKGRFTISRDNAKKKVYLQMNSLKPEDTAVYYCNV

SEQ ID NO: 153 - protein, 11 aa, artificial sequence
  10G11 and 10E11 Framework region 4
WGQGTQVTVSS

SEQ ID NO: 154 - protein, 25 aa, artificial sequence
  10E11? Framework region 1 (Q)
QVQLQESGGGLVQAGGSLRLSCAAS

SEQ ID NO: 155 - protein, 25 aa, artificial sequence
  10E11? Framework region 1 (D)
DVQLQESGGGLVQAGGSLRLSCAAS

SEQ ID NO: 156 - protein, 14 aa, artificial sequence
  10E11? Framework region 2
WYRQAPGKERELVA

SEQ ID NO: 157 - protein, 39 aa, artificial sequence
  10E11? Framework region 3
YADSVKGRFTISRGNAKNTVYLQMSSLKPEDTAVYYCNA

SEQ ID NO: 158 - protein, 25 aa, artificial sequence
  12C03 Framework region 1 (Q)
QVQLQESGGGLVQAGDSLRLSCAAS

SEQ ID NO: 159 - protein, 25 aa, artificial sequence
  12C03 Framework region 1 (D)
DVQLQESGGGLVQAGDSLRLSCAAS

SEQ ID NO: 160 - protein, 16 aa, artificial sequence
  12C03 Framework region 2
MGWFRQPPGKEREFVA

SEQ ID NO: 161 - protein, 39 aa, artificial sequence
  12C03 Framework region 3
YADSVKGRFTISRDNAMNTVYLQMNSLKPEDTAVYYCAA